European Patent Specification EP 3 770 237 B1, published June 11, 2025. Title: Wasch- und Reinigungsmittel mit verbesserter Enzym-Stabilität. Applicant: Henkel AG & Co. KGaA. The sequence listing filed with the application follows.

SEQUENCE LISTING (20 sequences)

SEQ ID NO: 1 - protein, 269 aa, Bacillus gibsonii
QQTVPWGITRVQAPTVHNRGITGSGVKVAILDTGIAQHSDLTIRGGASFVPGESTTADLNGHGTHVAGTVAALNNSIGVIGVAPSADLYAVKVLGANGRGSVSGIAQGLEWAATNNMHIANMSLGSDAPSTTLERAVNYATSRGVLVIAATGNNGTGSIGYPARYANAMAVGATDQNNRRASFSQYGTGIDIVAPGVGIQSTYLNNSYASMPGTSMATPHVAGVAALVKQKNPSWNATQIRNHLKNTATNLGNSSQFGSGLVNADAATR

SEQ ID NO: 2 - protein, 4 aa, artificial sequence
  enzyme stabilizer
  MOD_RES (1)..(1): Ac-Leu, Ac-Phe, Ac-Tyr
XGAY

SEQ ID NO: 3 - protein, 4 aa, artificial sequence
  enzyme stabilizer
  MOD_RES (1)..(1): Ac-Phe
XGAL

SEQ ID NO: 4 - protein, 4 aa, artificial sequence
  enzyme stabilizer
  MOD_RES (1)..(1): Ac-Phe
XGAF

SEQ ID NO: 5 - protein, 4 aa, artificial sequence
  enzyme stabilizer
  MOD_RES (1)..(1): Ac-Phe
XGVY

SEQ ID NO: 6 - protein, 4 aa, artificial sequence
  enzyme stabilizer
  MOD_RES (1)..(1): Ac-Phe
XGAM

SEQ ID NO: 7 - protein, 4 aa, artificial sequence
  enzyme stabilizer
  MOD_RES (1)..(1): Ac-Trp
XLVY

SEQ ID NO: 8 - protein, 4 aa, artificial sequence
  enzyme stabilizer
  MOD_RES (1)..(1): MeO-CO-Phe, MeSO2-Phe, EtSO2-Phe, MeO(OH)(O)P-Leu
XGAL

SEQ ID NO: 9 - protein, 4 aa, artificial sequence
  enzyme stabilizer
  MOD_RES (1)..(1): MeO-CO-Phe
XGAF

SEQ ID NO: 10 - protein, 5 aa, artificial sequence
  enzyme stabilizer
  MISC_FEATURE (2)..(2): urea
FXRVY

SEQ ID NO: 11 - protein, 5 aa, artificial sequence
  enzyme stabilizer
  MISC_FEATURE (2)..(2): urea
FXGGY

SEQ ID NO: 12 - protein, 5 aa, artificial sequence
  enzyme stabilizer
  MISC_FEATURE (2)..(2): urea
FXGAF

SEQ ID NO: 13 - protein, 5 aa, artificial sequence
  enzyme stabilizer
  MISC_FEATURE (2)..(2): urea
FXGAY

SEQ ID NO: 14 - protein, 5 aa, artificial sequence
  enzyme stabilizer
  MISC_FEATURE (2)..(2): urea
FXGAL

SEQ ID NO: 15 - protein, 5 aa, artificial sequence
  enzyme stabilizer
  MISC_FEATURE (2)..(2): urea
  MISC_FEATURE (5)..(5): Nva, Nle
FXGAX

SEQ ID NO: 16 - protein, 5 aa, artificial sequence
  enzyme stabilizer
  MISC_FEATURE (2)..(2): urea
YXRVY

SEQ ID NO: 17 - protein, 5 aa, artificial sequence
  enzyme stabilizer
  MISC_FEATURE (2)..(2): urea
YXGAY

SEQ ID NO: 18 - protein, 6 aa, artificial sequence
  enzyme stabilizer
FCSRVF

SEQ ID NO: 19 - protein, 6 aa, artificial sequence
  enzyme stabilizer
FCSRVY

SEQ ID NO: 20 - protein, 6 aa, artificial sequence
  enzyme stabilizer
FCSGAY